European Patent Specification EP 3 487 521 B1, published September 2, 2026. Title: Ebola Virus Antibodies and Binding Agents Derived Therefrom. Applicant: Emory University Ahmed, Rafi. The sequence listing filed with the application follows.

SEQUENCE LISTING (214 sequences)

SEQ ID NO: 1 - protein, 107 aa, Artificial
  Synthetic
DIQMTQSPSSLSASVGDRVTITCRASQSISSFLNWHQQKPGKAPKLLIYAASSLQSGVPSRFSGSGSGTDFTLTISSLQPEDFAIYYCQQSYISPFTFGPGTKVDIK

SEQ ID NO: 2 - protein, 118 aa, Artificial
  Synthetic
EVQLVESGGGLVQPGGSLRLSCAASGFTFRSYDMHWVRQATGKGLEWVSAIGTAGDTYYPGSVKGRFTISRENAKNSLYLQMNSLRAEDTAVYYCARVRFGDTAVDYWGQGTLVTVSS

SEQ ID NO: 3 - protein, 113 aa, Artificial
  Synthetic
DIVMTQSPRSLSVTPGEPASISCRSSQSLLHRNGYNYLDWYLQKPGQSPQLLIYLGSNRASGVPDRFSGSGSGTDFTLKISRVEAEDVGVYYCMQALQTPSWTFGQGTKVEIK

SEQ ID NO: 4 - protein, 122 aa, Artificial
  Synthetic
EVQLVESGGGLIQPGGSLRLSCAASGFAVRSNYLSWVRQAPGKGLEWVSLIYSGGLTAYADSVEGRFTISRDNSKNTLYLQMNSLRVEDTALYYCARVASSAGTFYYGMDVWGQGTTVTVSS

SEQ ID NO: 5 - protein, 112 aa, Artificial
  Synthetic
QSVLTQPPSVSGAPGQRVTISCTGSSSNIGAGYDVYWYQQLPGTAPKLLIYGNSNRPSGVPDRFSGSKSGTSASLAITGLQAEDEADYYCQSFDSSLRDSWVFGGGTKLTVL

SEQ ID NO: 6 - protein, 120 aa, Artificial
  Synthetic
EVQLVESGGGLVKPGGSLRLSCAASGFTFSNAWMNWVRQAPGKGLEWVGRIKSKTDGGAADYAAPVKGRFTISRDDSKNTLYLQMNSLKTEDTAVYFCTTVYRYNYDSVWGQGTLVTVSS

SEQ ID NO: 7 - protein, 108 aa, Artificial
  Synthetic
EIVLTQSPGTLSLSPGERATLSCRASQSVSSSYLAWYQQKPGQAPRLLIYGAFNRATGIPDRFSGSGSGTDFTLTISRLEPEDFAVYYCQLYGSSPWTFGQGTKVEIK

SEQ ID NO: 8 - protein, 120 aa, Artificial
  Synthetic
EVQLLESGGGLVQPGGSLRLSCAASGFTFSTYGMSWVRQAPGKGLEWVSGISGSGGITYYADSVRGRFTISRDNSKNTLYLRMNSLRAEDTAVYYCAKVGEYYDFWSGYSPFEYWGQGTL

SEQ ID NO: 9 - protein, 108 aa, Artificial
  Synthetic
DIQMTQSPSTLSASVGDRVTITCRASQRINNLVAWYQQKPGKAPKVMIYDASSLKSGVPSRFSGSGSGTEFTLTISSLQPDDFATYFCQQYDTDSGWTFGQGTKVEIK

SEQ ID NO: 10 - protein, 129 aa, Artificial
  Synthetic
EVQLLESGGGLVQPGGSLRLSCAASGFTFSKYAMIWVRQAPGKGLQWVAGINKSGGRTYYADSVRGRFTISRDNSKNTLYLQMKSLRADDTAMYYCAKEGSPLSDVLLVAAPFGWFDPWGQGTLVTVSS

SEQ ID NO: 11 - protein, 11 aa, Artificial
  Synthetic
RASQSISSFLN

SEQ ID NO: 12 - protein, 7 aa, Artificial
  Synthetic
AASSLQS

SEQ ID NO: 13 - protein, 9 aa, Artificial
  Synthetic
QQSYISPFT

SEQ ID NO: 14 - protein, 9 aa, Artificial
  Synthetic
FTFRSYDMH

SEQ ID NO: 15 - protein, 10 aa, Artificial
  Synthetic
IGTAGDTYYP

SEQ ID NO: 16 - protein, 10 aa, Artificial
  Synthetic
VRFGDTAVDY

SEQ ID NO: 17 - protein, 16 aa, Artificial
  Synthetic
RSSQSLLHRNGYNYLD

SEQ ID NO: 18 - protein, 7 aa, Artificial
  Synthetic
LGSNRAS

SEQ ID NO: 19 - protein, 10 aa, Artificial
  Synthetic
MQALQTPSWT

SEQ ID NO: 20 - protein, 9 aa, Artificial
  Synthetic
FAVRSNYLS

SEQ ID NO: 21 - protein, 16 aa, Artificial
  Synthetic
LIYSGGLTAYADSVEG

SEQ ID NO: 22 - protein, 14 aa, Artificial
  Synthetic
VASSAGTFYYGMDV

SEQ ID NO: 23 - protein, 14 aa, Artificial
  Synthetic
TGSSSNIGAGYDVY

SEQ ID NO: 24 - protein, 7 aa, Artificial
  Synthetic
GNSNRPS

SEQ ID NO: 25 - protein, 12 aa, Artificial
  Synthetic
QSFDSSLRDSWV

SEQ ID NO: 26 - protein, 9 aa, Artificial
  Synthetic
FTFSNAWMN

SEQ ID NO: 27 - protein, 19 aa, Artificial
  Synthetic
RIKSKTDGGAADYAAPVKG

SEQ ID NO: 28 - protein, 9 aa, Artificial
  Synthetic
VYRYNYDSV

SEQ ID NO: 29 - protein, 12 aa, Artificial
  Synthetic
RASQSVSSSYLA

SEQ ID NO: 30 - protein, 7 aa, Artificial
  Synthetic
GAFNRAT

SEQ ID NO: 31 - protein, 9 aa, Artificial
  Synthetic
QLYGSSPWT

SEQ ID NO: 32 - protein, 9 aa, Artificial
  Synthetic
FTFSTYGMS

SEQ ID NO: 33 - protein, 17 aa, Artificial
  Synthetic
GISGSGGITYYADSVRG

SEQ ID NO: 34 - protein, 16 aa, Artificial
  Synthetic
VGEYYDFWSGYSPFEY

SEQ ID NO: 35 - protein, 11 aa, Artificial
  Synthetic
RASQRINNLVA

SEQ ID NO: 36 - protein, 7 aa, Artificial
  Synthetic
DASSLKS

SEQ ID NO: 37 - protein, 10 aa, Artificial
  Synthetic
QQYDTDSGWT

SEQ ID NO: 38 - protein, 9 aa, Artificial
  Synthetic
FTFSKYAMI

SEQ ID NO: 39 - protein, 17 aa, Artificial
  Synthetic
GINKSGGRTYYADSVRG

SEQ ID NO: 40 - protein, 20 aa, Artificial
  Synthetic
EGSPLSDVLLVAAPFGWFDP

SEQ ID NO: 41 - protein, 7 aa, Artificial
  Synthetic
  X (1)..(7): X is any amino acid
RXSQXIX

SEQ ID NO: 42 - protein, 6 aa, Artificial
  Synthetic
  X (1)..(6): X is any amino acid
RXSQSX

SEQ ID NO: 43 - protein, 6 aa, Artificial
  Synthetic
  X (1)..(6): X is any amino acid
ASSLXS

SEQ ID NO: 44 - protein, 6 aa, Artificial
  Synthetic
  X (1)..(6): X is any amino acid
XSNRXS

SEQ ID NO: 45 - protein, 9 aa, Artificial
  Synthetic
  X (1)..(9): X is any amino acid
QXXXXSPXT

SEQ ID NO: 46 - protein, 6 aa, Artificial
  Synthetic
  X (1)..(6): X is any amino acid
FXXRSX

SEQ ID NO: 47 - protein, 8 aa, Artificial
  Synthetic
  X (1)..(8): X is any amino acid
FTFXXYXM

SEQ ID NO: 48 - protein, 11 aa, Artificial
  Synthetic
  X (1)..(11): X is any amino acid
GXXXYXXSVXG

SEQ ID NO: 49 - protein, 10 aa, Artificial
  Synthetic
  X (1)..(10): X is any amino acid
VXXXXXXXXY

SEQ ID NO: 50 - protein, 328 aa, Homo sapiens
STKGPSVFPLAPSSKSTSGGTAALGCLVKDYFPEPVTVSWNSGALTSGVHTFPAVLQSSGLYSLSSVVTVPSSSLGTQTYICNVNHKPSNTKVDKKVEPKSCDKTHTCPPCPAPELLGGPSVFLFPPKPKDTLMISRTPEVTCVVVDVSHEDPEVKFNWYVDGVEVHNAKTKPREEQYNSTYRVVSVLTVLHQDWLNGKEYKCKVSNKALPAPIEKTISKAKGQPREPQVYTLPPSRDELTKNQVSLTCLVKGFYPSDIAVEWESNGQPENNYKTTPPVLDSDGSFFLYSKLTVDKSRWQQGNVFSCSVMHEALHNHYTQKSLSLSPG

SEQ ID NO: 51 - DNA, 321 bp, Artificial
  Synthetic
gacatccagatgacccagtctccatcctccctgtctgcatctgtaggagacagagtcaccatcacttgccgggcaagtcagagcattagcagctttttaaattggcatcagcagaaaccagggaaagcccctaagctcctgatctatgctgcatccagtttgcaaagtggggtcccatcaaggttcagtggcagtggatctgggacagatttcactctcaccatcagcagtctgcaacctgaagattttgcaatttactactgtcaacagagttacatttccccattcactttcggccctgggaccaaagtggatatcaaa

SEQ ID NO: 52 - DNA, 356 bp, Artificial
  Synthetic
gaggtgcagctggtggagtctgggggaggcttggtacagcctggggggtccctgagactctcctgtgcagcctctggattcaccttcagaagctacgacatgcactgggtccgccaagctacaggaaaaggtctggagtgggtctcagctattggtactgctggtgacacatactatccaggctccgtgaagggccgattcaccatctccagagaaaatgccaagaactccttgtatcttcaaatgaacagcctgagagccgaggacacggccgtgtattactgtgcaagagtccgtttcggggatacagccgttgactactggggccagggaaccctggtcaccgtctcctcagc

SEQ ID NO: 53 - DNA, 339 bp, Artificial
  Synthetic
gatattgtgatgactcagtctccacgctccctgtccgtcacccctggagagccggcctccatctcctgcaggtctagtcagagcctcctgcatagaaatggatataactatttggattggtatctgcagaagccagggcagtctccacagctcctgatctatttgggttctaatcgggcctccggggtccctgacaggttcagtggcagtggatcaggcacagattttacactgaaaatcagcagagtggaggctgaagatgttggggtttattactgcatgcaagctctacaaactccctcgtggacgttcggccaagggaccaaggtggaaatcaaa

SEQ ID NO: 54 - DNA, 368 bp, Artificial
  Synthetic
gaggtgcagctggtggagtcaggaggaggcttgatccagcctggggggtccctgagactctcctgtgcagcctctggtttcgccgtcaggagcaactacttgagctgggtccgccaggctcctgggaaggggctggagtgggtctcacttatttatagtggtggtctcacagcctacgcagactccgtggagggccggttcaccatctccagagacaattctaagaacacactatatcttcaaatgaacagcctgagagtcgaggacacggccctatattactgtgcgagagtcgcatcatcggctggaaccttctactacggtatggacgtctggggccaagggaccacggtcaccgtctcctcagc

SEQ ID NO: 55 - DNA, 336 bp, Artificial
  Synthetic
cagtctgtgctgacgcagccgccctcagtgtctggggccccagggcagagggtcaccatctcctgcactgggagcagttccaacatcggggcaggttatgatgtatactggtaccagcagcttccaggaacagcccccaaactcctcatctatggtaacagcaatcggccctcaggggtccctgaccgattctctggctccaagtctggcacctcagcctccctggccatcactgggctccaggctgaggatgaggctgattactactgccagtcctttgacagcagcctgagagattcttgggtgttcggcggggggaccaagctgaccgtccta

SEQ ID NO: 56 - DNA, 362 bp, Artificial
  Synthetic
gaggtgcagctggtggagtctgggggaggcttggtaaaacctggggggtcccttagactctcctgtgcagcctctggattcactttcagtaacgcctggatgaactgggtccgccaggctccagggaaggggctggagtgggttggccgtattaagagcaaaactgatggtggggctgcagactacgctgcacccgtgaagggcagattcaccatctcaagagatgattcaaaaaacacgctgtatctgcaaatgaacagcctgaaaaccgaggacacagccgtgtatttctgtaccacagtctacagatacaactatgattccgtctggggccagggaaccctggtcaccgtctcctcagc

SEQ ID NO: 57 - DNA, 324 bp, Artificial
  Synthetic
gaaattgtgttgacgcagtctccaggcaccctgtctttgtctccaggggaaagagccaccctctcctgcagggccagtcagagtgttagcagcagctacttagcctggtaccagcagaaacctggccaggctcccaggctcctcatctatggtgcatttaacagggccactggcatcccagacaggttcagtggcagtgggtctgggacagacttcactctcaccatcagcagactggagcctgaagattttgcagtgtattactgtcagctgtatggtagctcaccgtggacgttcggccaagggaccaaggtggaaatcaaa

SEQ ID NO: 58 - DNA, 377 bp, Artificial
  Synthetic
gaggtgcagctgttggagtctgggggaggcttggtacagcctggggggtccctgagactctcctgtgcagcctctggattcacctttagcacctatggcatgagctgggtccgccaggctccagggaaggggctggagtgggtctcaggtattagtggtagtggtggtatcacatactacgcagactccgtgaggggccggttcaccatctccagagacaattccaagaacacgctgtatctgcgaatgaacagcctgagagccgaggacacggccgtatattactgtgcgaaagtgggggagtattacgatttttggagtggttattccccctttgaatactggggccagggaaccctggtcaccgtctcctcagc

SEQ ID NO: 59 - DNA, 324 bp, Artificial
  Synthetic
gacatccagatgacccagtctccttccaccctgtctgcatctgtaggagacagagtcaccatcacttgccgggccagtcagaggattaataatttggtggcctggtatcagcagaaaccagggaaagcccctaaggtcatgatctatgatgcctccagtttgaaaagtggggtcccatcaaggttcagcggcagtggatctgggacagaattcactctcaccatcagcagcctgcaacctgatgattttgcaacttatttctgccaacagtatgatactgattcggggtggacgttcggccaagggaccaaggtggaaatcaaa

SEQ ID NO: 60 - DNA, 389 bp, Artificial
  Synthetic
gaggtgcagctgttggagtctgggggaggcctggtacagccgggggggtccctgagactctcctgtgccgcctctggattcacctttagcaaatatgccatgatctgggtccgccaggccccagggaaggggctgcagtgggtcgcaggtattaataagagtggtggcaggacatactacgcagactccgtgaggggccggttcaccatctccagagacaattccaagaatacgctgtacctgcaaatgaaaagcctgagagccgacgacacggccatgtattactgtgcgaaagagggatcccctttatcagatgttttactggtagcagctccatttgggtggttcgatccctggggccagggaaccctggtcaccgtctcctcagc

SEQ ID NO: 61 - protein, 16 aa, Artificial
  Synthetic
  X (1)..(16): X is any amino acid
YXXLXXXXXXXXYXXL

SEQ ID NO: 62 - protein, 150 aa, Artificial
  Synthetic
AQLPITEAQSFGLLDPKLCYLLDGILFIYGVILTALFLRVKFSRSADAPAYQQGQNQLYNELNLGRREEYDVLDKRRGRDPEMGGKPRRKNPQEGLYNELQKDKMAEAYSEIGMKGERRRGKGHDGLYQGLSTATKDTYDALHMQALPPR

SEQ ID NO: 63 - protein, 151 aa, Artificial
  Synthetic
AQLPITEAQSFGLLDPKLCYLLDGILFIYGVILTALFLRVKFSRSADAPAYQQGQNQLYNELNLGRREEYDVLDKRRGRDPEMGGKPQRRKNPQEGLYNELQKDKMAEAYSEIGMKGERRRGKGHDGLYQGLSTATKDTYDALHMQALPPR

SEQ ID NO: 64 - protein, 150 aa, Artificial
  Synthetic
AQLPITEAQSFGLLDPKLCYLLDGILFIYGVILTALFLRVKFSRSAEPPAYQQGQNQLYNELNLGRREEYDVLDKRRGRDPEMGGKPRRKNPQEGLYNELQKDKMAEAYSEIGMKGERRRGKGHDGLYQGLSTATKDTYDALHMQALPPR

SEQ ID NO: 65 - protein, 62 aa, Artificial
  Synthetic
EPQLCYILDAILFLYGIVLTLLYCRLKIQVRKAAITSYEKSDGVYTGLSTRNQETYETLKHE

SEQ ID NO: 66 - protein, 330 aa, Artificial
  Synthetic
RSTKGPSVFPLAPSSKSTSGGTAALGCLVKDYFPEPVTVSWNSGALTSGVHTFPAVLQSSGLYSLSSVVTVPSSSLGTQTYICNVNHKPSNTKVDKKVEPKSCDKTHTCPPCPAPELLGGPSVFLFPPKPKDTLMISRTPEVTCVVVDVSHEDPEVKFNWYVDGVEVHNAKTKPREEQYNSTYRVVSVLTVLHQDWLNGKEYKCKVSNKALPAPIEKTISKAKGQPREPQVYTLPPSRDELTKNQVSLTCLVKGFYPSDIAVEWESNGQPENNYKTTPPVLDSDGSFFLYSKLTVDKSRWQQGNVFSCSVMHEALHNHYTQKSLSLSPGK

SEQ ID NO: 67 - protein, 330 aa, Artificial
  Synthetic
RSTKGPSVFPLAPSSKSTSGGTAALGCLVKDYFPEPVTVSWNSGALTSGVHTFPAVLQSSGLYSLSSVVTVPSSSLGTQTYICNVNHKPSNTKVDKKVEPKSCDKTHTCPPCPAPELLGGPSVFLFPPKPKDTLMISRTPEVTCVVVDVSHEDPEVKFNWYVDGVEVHNAKTKPREEQYASTYRVVSVLTVLHQDWLNGKEYKCKVSNKALPAPIEKTISKAKGQPREPQVYTLPPSRDELTKNQVSLTCLVKGFYPSDIAVEWESNGQPENNYKTTPPVLDSDGSFFLYSKLTVDKSRWQQGNVFSCSVMHEALHNHYTQKSLSLSPGK

SEQ ID NO: 68 - protein, 330 aa, Artificial
  Synthetic
RSTKGPSVFPLAPSSKSTSGGTAALGCLVKDYFPEPVTVSWNSGALTSGVHTFPAVLQSSGLYSLSSVVTVPSSSLGTQTYICNVNHKPSNTKVDKKVEPKSCDKTHTCPPCPAPELLGGPSVFLFPPKPKDTLYITREPEVTCVVVDVSHEDPEVKFNWYVDGVEVHNAKTKPREEQYNSTYRVVSVLTVLHQDWLNGKEYKCKVSNKALPAPIEKTISKAKGQPREPQVYTLPPSRDELTKNQVSLTCLVKGFYPSDIAVEWESNGQPENNYKTTPPVLDSDGSFFLYSKLTVDKSRWQQGNVFSCSVMHEALHNHYTQKSLSLSPGK

SEQ ID NO: 69 - protein, 108 aa, Artificial
  Synthetic
EIVLTQSPGTLSLSPGERATLSCRASQSVSSSYLAWYQQKPGQAPRLLIYGAFNRATGIPDRFSGSGSGTDFTLTISRLEPEDFAVYYCQQYGRSPFTFGPGTKVDIK

SEQ ID NO: 70 - protein, 7 aa, Artificial
  Synthetic
QSVSSSY

SEQ ID NO: 71 - protein, 7 aa, Artificial
  Synthetic
GAFNRAT

SEQ ID NO: 72 - protein, 9 aa, Artificial
  Synthetic
QQYGRSPFT

SEQ ID NO: 73 - protein, 125 aa, Artificial
  Synthetic
EVQLVESGGGLVQPGGSLRLSCAASGFAFSTYAMSWVRQAPGKGLEWVSAITGSGYSTYYADSVKGRFTISGDNSKNTLYLQMNSLRAEDTALYYCAKVGEYYDFWSGYSPFDSWGQGTLVTVSS

SEQ ID NO: 74 - protein, 8 aa, Artificial
  Synthetic
GFAFSTYA

SEQ ID NO: 75 - protein, 8 aa, Artificial
  Synthetic
ITGSGYST

SEQ ID NO: 76 - protein, 18 aa, Artificial
  Synthetic
AKVGEYYDFWSGYSPFDS

SEQ ID NO: 77 - protein, 112 aa, Artificial
  Synthetic
DIVMTQTPLSSAVTLGQPASISCRSSQRLVHSDGNTYLSWLHQRPGQPPRLLIYKVSLRFSGVPDRFSGSGAGTDFTLKISRVEAEDVGIYYCMQATQFPLTFGGGTKVEIK

SEQ ID NO: 78 - protein, 11 aa, Artificial
  Synthetic
QRLVHSDGNTY

SEQ ID NO: 79 - protein, 7 aa, Artificial
  Synthetic
KVSLRFS

SEQ ID NO: 80 - protein, 9 aa, Artificial
  Synthetic
MQATQFPLT

SEQ ID NO: 81 - protein, 115 aa, Artificial
  Synthetic
EVQLLESGGGLVKPGGSLRLSCAASGFTFNEYMMNWVRQPPGKGLEWVSSISGTSTYINYADSVKGRFTISRDNAKNSLYLQMNSLRSDDTAMYYCARGSTGGYWGQGTLITVSS

SEQ ID NO: 82 - protein, 8 aa, Artificial
  Synthetic
GFTFNEYM

SEQ ID NO: 83 - protein, 8 aa, Artificial
  Synthetic
ISGTSTYI

SEQ ID NO: 84 - protein, 6 aa, Artificial
  Synthetic
GSTGGY

SEQ ID NO: 85 - protein, 107 aa, Artificial
  Synthetic
DIQMTQSPSSLSASVGDRVTITCRASQSISSYLNWYQQKPGKAPKVLIYSAFSLQNGVPSRFSGSGSGTDFTLTISSLQPEDFATYYCQQSYSTPRTFGQGTKVEIK

SEQ ID NO: 86 - protein, 8 aa, Artificial
  Synthetic
QSISSYLN

SEQ ID NO: 87 - protein, 7 aa, Artificial
  Synthetic
SAFSLQN

SEQ ID NO: 88 - protein, 9 aa, Artificial
  Synthetic
QQSYSTPRT

SEQ ID NO: 89 - protein, 116 aa, Artificial
  Synthetic
QVQLQESGPGLVKPSGTLSLTCAVSGGSISSTNWWSWVRQPPGKGLEWIGEIYHSGSTNYNPSLKSRVTISLDKSKDQFSLKLSSVTAADTAVYYCAYSNTWTGGWGQGTLVTVSS

SEQ ID NO: 90 - protein, 10 aa, Artificial
  Synthetic
GSISSTNWWS

SEQ ID NO: 91 - protein, 6 aa, Artificial
  Synthetic
HSGSTN

SEQ ID NO: 92 - protein, 7 aa, Artificial
  Synthetic
SNTWTGG

SEQ ID NO: 93 - protein, 107 aa, Artificial
  Synthetic
EVVLTQSPVTLSLSPGERATLSCRASQSVSGYLAWYQQKPGQVPRLLIYDTSNRATGIPARFSGSGSGTDFTLTISTIEPEDFAVYYCQQRSKWGVTFGGGTKVDIK

SEQ ID NO: 94 - protein, 8 aa, Artificial
  Synthetic
QSVSGYLA

SEQ ID NO: 95 - protein, 7 aa, Artificial
  Synthetic
DTSNRAT

SEQ ID NO: 96 - protein, 9 aa, Artificial
  Synthetic
QQRSKWGVT

SEQ ID NO: 97 - protein, 124 aa, Artificial
  Synthetic
QVQLVQSGAEVKKPGASVNLSCKGSGYSFRTYYIHWVRQAPGQGLEWMGIINSSGGGTTYAQKFQGRVTMTRDTSTSTVYMELRSLKYEDTAMYYCARDRFPTVSGEPFAMDVWGQGTTVTVSS

SEQ ID NO: 98 - protein, 10 aa, Artificial
  Synthetic
GYSFRTYYIH

SEQ ID NO: 99 - protein, 10 aa, Artificial
  Synthetic
INSSGGGTTY

SEQ ID NO: 100 - protein, 15 aa, Artificial
  Synthetic
DRFPTVSGEPFAMDV

SEQ ID NO: 101 - protein, 109 aa, Artificial
  Synthetic
EIVLTQSPGTLSLSPGERATLSCRASQSVTSNYLAWYQQKPGQAPRVLIYGASSRATGIPDRFSGSGSGTDFTLTISRLEPEDFAVYYCQQFGASPPYSFGQGTKVEIK

SEQ ID NO: 102 - protein, 9 aa, Artificial
  Synthetic
QSVTSNYLA

SEQ ID NO: 103 - protein, 7 aa, Artificial
  Synthetic
GASSRAT

SEQ ID NO: 104 - protein, 10 aa, Artificial
  Synthetic
QQFGASPPYS

SEQ ID NO: 105 - protein, 127 aa, Artificial
  Synthetic
EVQLVESGGGLIQPGGSLRLSCTASGFTFSKFAMSWVRQAPGRGLEWISYISGGSKTKYYADSVRGRFTISRDNAKGSLFLQMNSLRAEDTAIYFCAKKGWQSTFLGMDYFYGMDVWGKGTTVTVSS

SEQ ID NO: 106 - protein, 10 aa, Artificial
  Synthetic
GFTFSKFAMS

SEQ ID NO: 107 - protein, 9 aa, Artificial
  Synthetic
ISGGSKTKY

SEQ ID NO: 108 - protein, 20 aa, Artificial
  Synthetic
AKKGWQSTFLGMDYFYGMDV

SEQ ID NO: 109 - protein, 113 aa, Artificial
  Synthetic
DIVMTQSPDSLAVSLGERASINCKSSQSVLSSSNTKNYLAWYQHKPGQPPKLLIYWASTRESGVPDRFSGSGSGTDFTLTISSLQPEDVAVYYCQQYYGAPYTFGQGTKVEIK

SEQ ID NO: 110 - protein, 12 aa, Artificial
  Synthetic
QSVLSSSNTKNY

SEQ ID NO: 111 - protein, 7 aa, Artificial
  Synthetic
WASTRES

SEQ ID NO: 112 - protein, 9 aa, Artificial
  Synthetic
QQYYGAPYT

SEQ ID NO: 113 - protein, 118 aa, Artificial
  Synthetic
EVQLVESGGGLVQPGGSLRLSCAASGFTFRSYDMDWFRQSTGKGLEWVSAIGSAGDTYYTDSVKGRFTISRENGKNSLYLQMNSLRAGDTAVYYCARARFGDNVFDLWGRGTLVTVSS

SEQ ID NO: 114 - protein, 9 aa, Artificial
  Synthetic
FTFRSYDMD

SEQ ID NO: 115 - protein, 7 aa, Artificial
  Synthetic
IGSAGDT

SEQ ID NO: 116 - protein, 10 aa, Artificial
  Synthetic
ARFGDNVFDL

SEQ ID NO: 117 - protein, 108 aa, Artificial
  Synthetic
EIVLTQSPGTLSLSPGERAALSCRASQSVSGNYFAWYQQKSGQAPRLLISAASSRATGVPDRFSASGSGTDFTLTISRLEPEDSAVYYCQQYGSSPLTFGQGTKVEIK

SEQ ID NO: 118 - protein, 8 aa, Artificial
  Synthetic
SVSGNYFA

SEQ ID NO: 119 - protein, 7 aa, Artificial
  Synthetic
AASSRAT

SEQ ID NO: 120 - protein, 9 aa, Artificial
  Synthetic
QQYGSSPLT

SEQ ID NO: 121 - protein, 118 aa, Artificial
  Synthetic
EVQLVQSGGGLAQPGGSLRLSCAASGFTFRSYDMHWVRQVTGKGLEWVSAIGTAGDTYYTGSVKGRFTISRENDKSSLYLQMSSLRGEDTAVYYCARAAFGSHYFDYWGQGTLVTVSS

SEQ ID NO: 122 - protein, 9 aa, Artificial
  Synthetic
FTFRSYDMH

SEQ ID NO: 123 - protein, 10 aa, Artificial
  Synthetic
IGTAGDTYYT

SEQ ID NO: 124 - protein, 10 aa, Artificial
  Synthetic
AAFGSHYFDY

SEQ ID NO: 125 - protein, 108 aa, Artificial
  Synthetic
SYELTQPPSVSVSPGQTARITCSGDALPKQYAYWYQQKPGQAPVPVIYKDSERPSGIPERFSGSSSGTTVTLTISGVQAEDEADYYCQSSDSSGTYVVFGGGTKLTVL

SEQ ID NO: 126 - protein, 6 aa, Artificial
  Synthetic
ALPKQY

SEQ ID NO: 127 - protein, 4 aa, Artificial
  Synthetic
KDSE

SEQ ID NO: 128 - protein, 11 aa, Artificial
  Synthetic
QSSDSSGTYVV

SEQ ID NO: 129 - protein, 120 aa, Artificial
  Synthetic
EVQLVQSGAEVKKPGASVKVSCKASGYTFTSYYMHWVRQAPGQGLEWMGIINPSGGSTSYAQKFQGRVTMTRDTSTSTVYMELSSLRSEDTAVYYCARHDSSGYDAFDIWGQGTMVTVSS

SEQ ID NO: 130 - protein, 8 aa, Artificial
  Synthetic
GYTFTSYY

SEQ ID NO: 131 - protein, 8 aa, Artificial
  Synthetic
INPSGGST

SEQ ID NO: 132 - protein, 13 aa, Artificial
  Synthetic
ARHDSSGYDAFDI

SEQ ID NO: 133 - protein, 112 aa, Artificial
  Synthetic
DIVMTQSPLSLPVTPGEPASISCRSSQSLLHSNGYNYVDWYLQKPGQSPQLLIYLGSSRASGVPDRFSGSGSGTDFTLKISRVETEDVGIYYCMQGLQTPLTFGGGTKVEIK

SEQ ID NO: 134 - protein, 11 aa, Artificial
  Synthetic
QSLLHSNGYNY

SEQ ID NO: 135 - protein, 4 aa, Artificial
  Synthetic
LGSS

SEQ ID NO: 136 - protein, 9 aa, Artificial
  Synthetic
MQGLQTPLT

SEQ ID NO: 137 - protein, 121 aa, Artificial
  Synthetic
QVQLVQSGAEVKKPGASVKVSCRTSGYTFSSYNIHWVRQAPGQGLEWMGVINPYGRSTTLYARRFRDRVTMTRDTSTSTVYMELSSLRSEDTAVYFCGRLYSGAPYGLDVWGQGSTVTVSS

SEQ ID NO: 138 - protein, 10 aa, Artificial
  Synthetic
GYTFSSYNIH

SEQ ID NO: 139 - protein, 7 aa, Artificial
  Synthetic
PYGRSTT

SEQ ID NO: 140 - protein, 13 aa, Artificial
  Synthetic
GRLYSGAPYGLDV

SEQ ID NO: 141 - protein, 113 aa, Artificial
  Synthetic
DIVLTQSPDSLAASLGERATISCKSSHSVLYSSNNKDFFAWYQQKPGQPPKLLISWASTRESGVPVRFNGGGSGTHFTLTISSLQAEDVAVYYCQQYFSSPITFGQGTRLEIK

SEQ ID NO: 142 - protein, 12 aa, Artificial
  Synthetic
HSVLYSSNNKDF

SEQ ID NO: 143 - protein, 4 aa, Artificial
  Synthetic
WAST

SEQ ID NO: 144 - protein, 9 aa, Artificial
  Synthetic
QQYFSSPIT

SEQ ID NO: 145 - protein, 124 aa, Artificial
  Synthetic
QVQLVQSGAEVKKPGSSVKVACKVSGGTFSSYTISWVRQAPGQGLEWMGGIIPSFGVGHYSQKFRDRVTLTADKSTTTAFLELSSVRSEDTALYYCAILGTFNWKSGGNYFGPWGQGTLVTVSS

SEQ ID NO: 146 - protein, 8 aa, Artificial
  Synthetic
GGTFSSYT

SEQ ID NO: 147 - protein, 8 aa, Artificial
  Synthetic
IIPSFGVG

SEQ ID NO: 148 - protein, 17 aa, Artificial
  Synthetic
AILGTFNWKSGGNYFGP

SEQ ID NO: 149 - protein, 107 aa, Artificial
  Synthetic
EIVLTQSPNTLSLSPGERATLSCRASQSLRTNQLAWYQQKPGQAPRLLIHTSTRATGIPDRFSGSGSGTDFTLTISGLEAEDFAVYYCQASDTSSLTFGGGTKLEIR

SEQ ID NO: 150 - protein, 6 aa, Artificial
  Synthetic
QSLRTN

SEQ ID NO: 151 - protein, 4 aa, Artificial
  Synthetic
HTST

SEQ ID NO: 152 - protein, 9 aa, Artificial
  Synthetic
QASDTSSLT

SEQ ID NO: 153 - protein, 125 aa, Artificial
  Synthetic
QVQLQESGPGLVKPSESLSLTCTISGGSIRDYYWSWIRQAPGKGLEWIGYKYHAARGNSNPSLESRVTMSIDTSRSEFSLRLTSVTAADTAVYYCARVQYGPGGGYYSGNWLDLWGQGTLVTVSS

SEQ ID NO: 154 - protein, 8 aa, Artificial
  Synthetic
GGSIRDYY

SEQ ID NO: 155 - protein, 7 aa, Artificial
  Synthetic
KYHAARG

SEQ ID NO: 156 - protein, 19 aa, Artificial
  Synthetic
ARVQYGPGGGYYSGNWLDL

SEQ ID NO: 157 - protein, 106 aa, Artificial
  Synthetic
EIVMTQSPATLSLSPGERASLSCRASQSIATNLAWYQQKPGQPPRVLIYGASTRATGIPTRFSGSGSGTEFTLTISSLQSEDFAIYYCHQYHSWRTFGQGTKVEMK

SEQ ID NO: 158 - protein, 6 aa, Artificial
  Synthetic
QSIATN

SEQ ID NO: 159 - protein, 4 aa, Artificial
  Synthetic
GAST

SEQ ID NO: 160 - protein, 8 aa, Artificial
  Synthetic
HQYHSWRT

SEQ ID NO: 161 - protein, 122 aa, Artificial
  Synthetic
QLQLQESGPGLVKPSETLSLTCTVSGGSVASSNDYWGWIRQPPGKGPEWIGTIFYRGTTDYNPSLKSRLTMSVDTSRNQFSLKLSSVTAADTAVYYCARLPLWFSELGHDYWGQGTLVTVSS

SEQ ID NO: 162 - protein, 10 aa, Artificial
  Synthetic
GGSVASSNDY

SEQ ID NO: 163 - protein, 7 aa, Artificial
  Synthetic
IFYRGTT

SEQ ID NO: 164 - protein, 14 aa, Artificial
  Synthetic
ARLPLWFSELGHDY

SEQ ID NO: 165 - protein, 111 aa, Artificial
  Synthetic
QSALTQPPSASGSPGQSVTISCTGTSSDVGVYNSVSWYRQHPGKVPKLMIYEVSKRPSGVPDRFSGSKSGNTASLTVSGLQADDEGDYYCCSCSGTNSLCVFGTGTKVTVL

SEQ ID NO: 166 - protein, 9 aa, Artificial
  Synthetic
SSDVGVYNS

SEQ ID NO: 167 - protein, 4 aa, Artificial
  Synthetic
EVSK

SEQ ID NO: 168 - protein, 11 aa, Artificial
  Synthetic
CSCSGTNSLCV

SEQ ID NO: 169 - protein, 124 aa, Artificial
  Synthetic
QVQLHESGPGLVQPSETLSLTCTVSGDSITNYYWSWIRQPPGKGLEWIGYMYYSASAHYNPSLQSRVTISVDTSKNQFSLKLSSVTAADTAVYFCARVDYSSSSYYSGNWFDPWGQGTLVTVSS

SEQ ID NO: 170 - protein, 8 aa, Artificial
  Synthetic
GDSITNYY

SEQ ID NO: 171 - protein, 7 aa, Artificial
  Synthetic
MYYSASA

SEQ ID NO: 172 - protein, 18 aa, Artificial
  Synthetic
ARVDYSSSSYYSGNWFDP

SEQ ID NO: 173 - protein, 112 aa, Artificial
  Synthetic
QSVLTQPPSVSGAPGQTVTISCTGSYSNIGAGYDVQWYQHLPGTAPKLLIYDNVHRPSGVPDRFSGSKSGTSASLAITGLQTEDEADYYCQSYDSRLRDQWVFGGGTKLTVL

SEQ ID NO: 174 - protein, 9 aa, Artificial
  Synthetic
YSNIGAGYD

SEQ ID NO: 175 - protein, 4 aa, Artificial
  Synthetic
DNVH

SEQ ID NO: 176 - protein, 12 aa, Artificial
  Synthetic
QSYDSRLRDQWV

SEQ ID NO: 177 - protein, 122 aa, Artificial
  Synthetic
EVQLVESGGDLVQPGGSLRLSCAASGITLSGVWMNWVRQAPGKGLEWIGRIKSTSDGGRADFAAPARGRFTMSRDESKNKLFLQMNNLGIEDTGMYYCFTRVQRDGTKDDFWGRGTLVTVSS

SEQ ID NO: 178 - protein, 8 aa, Artificial
  Synthetic
GITLSGVW

SEQ ID NO: 179 - protein, 10 aa, Artificial
  Synthetic
IKSTSDGGRA

SEQ ID NO: 180 - protein, 13 aa, Artificial
  Synthetic
FTRVQRDGTKDDF

SEQ ID NO: 181 - protein, 107 aa, Artificial
  Synthetic
QSALTQPASVSGSPGQSITLSCTVGGNKFVSWYQQHPGKAPKLIISDFTDRPSGVSSRFSGSKSGNTASLTISGLQPDDEATYFCSSYASTSTSLWVFGGGTKLTVL

SEQ ID NO: 182 - protein, 8 aa, Artificial
  Synthetic
CTVGGNKF

SEQ ID NO: 183 - protein, 4 aa, Artificial
  Synthetic
DFTD

SEQ ID NO: 184 - protein, 12 aa, Artificial
  Synthetic
SSYASTSTSLWV

SEQ ID NO: 185 - protein, 125 aa, Artificial
  Synthetic
QEQLQESGPGLVKPSGTLSLTCTVSGVSVSGSYFWNWVRQPPGKGLEWLGFIHSTGSTNTNPSLKSRVTISVDTSKNQFSLRLTSVSAADTAVYYCARAAWLVGGEYYNYGMDLWGQGTTVTVSS

SEQ ID NO: 186 - protein, 9 aa, Artificial
  Synthetic
GVSVSGSYF

SEQ ID NO: 187 - protein, 7 aa, Artificial
  Synthetic
IHSTGST

SEQ ID NO: 188 - protein, 18 aa, Artificial
  Synthetic
ARAAWLVGGEYYNYGMDL

SEQ ID NO: 189 - protein, 107 aa, Artificial
  Synthetic
GIQLTQSPSFLSASVGDRVTITCRASQGIYTYLAWYQQKPGKAPKLLVYVASTLQSGVPSRFSGSGSGTEFTLTISSLQPEDFATYYCQQLNSYPLTFGQGTKLEIK

SEQ ID NO: 190 - protein, 6 aa, Artificial
  Synthetic
QGIYTY

SEQ ID NO: 191 - protein, 4 aa, Artificial
  Synthetic
VASY

SEQ ID NO: 192 - protein, 9 aa, Artificial
  Synthetic
QQLNSYPLT

SEQ ID NO: 193 - protein, 127 aa, Artificial
  Synthetic
QVQLVESGGGVVQPGRSLRLSCVASGFTFSSYGMHWVRQAPGKGLEWVAFIWYDGTIQYYGDSVKGRFIISRDNSRNTLYLQMNSLRAEDTAVYYCASTLYRNGDYGSGSRTPDDYWGQGTLVTVSS

SEQ ID NO: 194 - protein, 8 aa, Artificial
  Synthetic
GFTFSSYG

SEQ ID NO: 195 - protein, 8 aa, Artificial
  Synthetic
IWYDGTIQ

SEQ ID NO: 196 - protein, 20 aa, Artificial
  Synthetic
ASTLYRNGDYGSGSRTPDDY

SEQ ID NO: 197 - DNA, 360 bp, Artificial
  Synthetic
gaggtgcagctggtgcagtctggggctgaggtgaagaagcctggggcctcagtgaaggtttcctgcaaggcatctggatacaccttcaccagctactatatgcactgggtgcgacaggcccctggacaagggcttgagtggatgggaataatcaaccctagtggtggtagcacaagctacgcacagaagttccagggcagagtcaccatgaccagggacacgtccacgagcacagtctacatggagctgagcagcctgagatctgaggacacggccgtgtattactgtgctaggcatgatagtagtggttatgatgcttttgatatctggggccaagggacaatggtcaccgtctcttca

SEQ ID NO: 198 - DNA, 324 bp, Artificial
  Synthetic
tcctatgagctgacacagccaccctcggtgtcagtgtccccaggacagacggccaggatcacctgctctggagatgcattgccaaagcaatatgcttattggtaccagcagaagccaggccaggcccctgtgccggtgatatataaagacagtgagaggccctcagggatccctgagcgattctctggctccagctcagggacaacagtcacgttgaccatcagtggagtccaggcagaagacgaggctgactattactgtcaatcatcagacagcagtggtacttatgtggtattcggcggagggaccaagctgaccgtccta

SEQ ID NO: 199 - DNA, 363 bp, Artificial
  Synthetic
caggtgcaactggtgcagtcaggggctgaggtgaagaagcctggggcctcagtgaaggtttcctgcaggacatctggatacacattctccagctacaatatacattgggtgcgacaggcccctggacaaggtcttgagtggatgggagttattaatccttatggccgtagtaccacactttacgcacggaggttccgggacagagtcaccatgaccagggacacgtccacgagcacagtttacatggaactgagcagcctgagatccgaggacacggccgtatacttctgtggaaggctttacagtggtgcaccctatggtttggacgtctggggccaagggagcacggtcaccgtctcttca

SEQ ID NO: 200 - DNA, 336 bp, Artificial
  Synthetic
gatattgtgatgactcagtctccactctccctgcccgtcacccctggagagccggcctccatctcctgcaggtctagtcagagcctcctgcatagtaatggatacaactatgtggattggtacctgcagaagccagggcagtctccacagctcctgatctatttgggttctagtcgggcctccggggtccctgacaggttcagtggcagtggatcaggcacagattttacactgaaaatcagcagagtggagactgaggatgttggcatttattactgcatgcaaggtctacaaactcccctcactttcggcggagggaccaaggtggagatcaaa

SEQ ID NO: 201 - DNA, 372 bp, Artificial
  Synthetic
caggtgcagctggtgcagtctggggctgaagtgaagaagcctgggtcctcggtgaaggtcgcctgcaaggtttctggaggcaccttcagcagctatactattagttgggtgcgacaggcccctggacaagggcttgagtggatgggagggatcatcccttcctttggtgtgggacactactcacagaagttccgggacagagtcacgctaaccgcggacaaatccacgaccacagccttcttggaactgagcagcgtgagatctgaagacacggccctatattactgtgcgatactggggacttttaactggaagtccgggggcaactacttcggcccctggggccaggggaccctggtcaccgtctcttca

SEQ ID NO: 202 - DNA, 339 bp, Artificial
  Synthetic
gacatcgtgctgacccagtctccagactccctggctgcgtctctgggcgagagggccaccatcagctgcaagtccagccacagtgttttatacagctccaacaataaggacttctttgcctggtaccagcagaaaccaggacagcctcccaaactgctcatttcctgggcatctacccgggaatccggggtccctgtccgattcaatggcggcgggtctgggacacatttcactctcaccatcagcagcctgcaggctgaagatgtggcagtttactactgtcagcaatattttagttctccgatcaccttcggccaagggacacgactggagattaaa

SEQ ID NO: 203 - DNA, 375 bp, Artificial
  Synthetic
caggtgcagctgcaggagtcgggcccaggactggtgaagccttcggagagcctgtccctcacatgcactatctctggcggctccataagggactattactggagctggattcggcaggccccagggaagggactggagtggatcggatataagtatcacgctgcgcgcggcaactccaatccctccctcgagagtcgagtcaccatgtccatcgacacgtccaggagcgagttctccctgaggctgacttctgtgaccgctgcggacacggccgtctattattgtgcgagagttcaatacggtcctgggggcggttactattcggggaactggttggacctctggggccagggaaccctggtcaccgtctcttca

SEQ ID NO: 204 - DNA, 321 bp, Artificial
  Synthetic
gaaattgtgttgacacagtctccaaacaccctgtctttgtctccaggggaaagagccaccctctcctgcagggccagtcagagtcttcgtaccaaccagttagcctggtaccagcaaaaacctggccaggctcccaggctcctcatccatacatccaccagggccactggcatcccagacaggttcagtggcagtgggtctgggacagacttcactctcaccatcagcggactggaggctgaagactttgcagtgtattactgtcaggcgtctgatacctcatcgctcactttcggcggagggaccaagttagagatcaga

SEQ ID NO: 205 - DNA, 366 bp, Artificial
  Synthetic
cagctgcagctgcaggagtcgggcccaggactggtgaagccttcggagaccctgtccctcacctgcactgtctctggtggctccgtcgccagtagtaatgactactggggctggatccgccagcccccagggaaggggccggagtggattgggactatcttttatagagggaccaccgactacaacccgtccctcaagagtcgactcactatgtccgtggacacgtccaggaaccagttctccctgaagctgagctctgtgaccgccgcagacacggctgtctattactgtgcgagactgcccctatggttcagtgagttaggtcatgactactggggccagggaaccctggtcaccgtctcctca

SEQ ID NO: 206 - DNA, 407 bp, Artificial
  Synthetic
gaaatagtgatgacgcagtctccagccaccctgtctctgtctccaggagaaagagcctccctgtcctgcagggccagtcagagtattgccaccaacttagcctggtaccagcaaaaacctggccagcctcccagggtcctcatctatggtgcatccacaagggcaactggtatcccaaccaggttcagtggcagtggatctgggacagagttcactctcaccatcagcagcctgcagtctgaagattttgcaatttattactgtcaccagtatcatagctggcggacgttcggccaagggaccaaggtagaaatgaaagtgcgagagtggactacagttcgagtagttattattcgggaaactggttcgacccctggggccagggaacccttgtcaccgtctcctca

SEQ ID NO: 207 - DNA, 372 bp, Artificial
  Synthetic
caggtgcagctgcatgagtcgggcccagggctggtgcagccttcggagaccctgtccctcacctgcactgtctctggtgactccatcactaattactactggagctggatccggcagcccccagggaagggactggagtggattggatatatgtattacagtgcgagcgcccactacaatccctccctccagagtcgagtcaccatttcagtggacacgtccaagaaccagttctccctgaaactgagctctgtgaccgctgcggacacggccgtgtatttctgtgcgagagtggactacagttcgagtagttattattcgggaaactggttcgacccctggggccagggaacccttgtcaccgtctcctca

SEQ ID NO: 208 - DNA, 333 bp, Artificial
  Synthetic
cagtctgccctgactcagcctccctccgcgtccgggtctcctggacagtcagtcaccatctcctgcactggaaccagcagtgacgttggtgtttataattctgtctcctggtaccgacagcacccaggcaaagtccccaaactcatgatttatgaggtcagtaagcggccctcaggggtccctgatcgcttctctggctccaagtccggcaacacggcctccctgaccgtctctgggctccaggctgacgatgagggtgattattactgctgctcatgttcaggcaccaacagcctctgtgtcttcggaactgggaccaaggtcaccgtcctg

SEQ ID NO: 209 - DNA, 366 bp, Artificial
  Synthetic
gaggtgcagctggtggagtctgggggagacttagtacagcctggggggtccctcagactctcctgtgcagcctctggaatcaccttgagtggagtttggatgaactgggtccgccaggctccagggaaggggctggagtggattggccgtattaaaagcacaagtgacggtgggagagcagacttcgccgcacccgcgagaggcagattcaccatgtcaagagatgagtcaaagaataagctgtttctgcaaatgaacaacctgggaatcgaagacacaggcatgtattattgtttcacgagagtccaaagagacggaactaaagatgacttctggggccggggaaccctggtcaccgtctcttca

SEQ ID NO: 210 - DNA, 336 bp, Artificial
  Synthetic
cagtctgtgctgacgcagccgccctcagtgtctggggccccagggcagacggtcaccatctcctgcactgggagctactccaacatcggggcaggttatgatgtacagtggtaccagcaccttcctggaacagcccccaaactcctcatttatgataatgtccatcggccctcaggggtccctgaccgattctctggctccaagtctggcacctcagcctccctggccatcactgggctccagactgaagatgaggctgattattattgccagtcctatgacagcagactgagggatcaatgggtgttcggcggagggaccaagctgaccgtccta

SEQ ID NO: 211 - DNA, 375 bp, Artificial
  Synthetic
caggagcagctgcaagagtcgggcccaggactggtgaagccttcggggaccctgtccctcacctgcactgtctccggcgtctccgtcagtgggagttacttctggaattgggtccgccagcccccagggaagggactggagtggcttggatttattcatagcactgggagcaccaacaccaacccctccctcaagagtcgagtcaccatttcagtagacacgtccaagaaccagttctccctgaggctgacttctgtgagcgctgcggacacggccgtttattactgtgcgagagccgcttggttagtagggggggagtactacaactacggtatggacctttggggccaagggaccacggttaccgtctcctca

SEQ ID NO: 212 - DNA, 321 bp, Artificial
  Synthetic
cagtctgccctgactcagcccgcctccgtttctgggtctcctggacagtcgatcaccctctcctgcactgtaggcggtaataagtttgtctcttggtatcaacaacacccaggcaaagcccccaaactcattatttctgatttcactgatcggccctcaggggtctctagtcgcttctctggctccaagtctggcaacacggcctccctgaccatctctgggctccagcctgacgacgaggctacttatttctgcagttcttacgcaagcaccagcacttctctttgggtcttcggcggggggaccaagctgaccgtccta

SEQ ID NO: 213 - DNA, 381 bp, Artificial
  Synthetic
caggtgcagctggtggaatctgggggaggcgtggtccagcctgggaggtccctgagactctcctgtgtagcgtctggattcaccttcagtagttatggcatgcactgggtccgccaggctccaggcaaggggctggagtgggtggcatttatatggtatgatggaactattcaatactatggagactccgtgaagggccgattcatcatctccagagacaattccaggaatacgctgtatctacaaatgaacagcctgagagccgaggacacggctgtgtattactgtgcgagcactctttaccgaaacggtgactacgggtcagggtcccggaccccggacgactactggggccagggaaccctggtcaccgtctcttca

SEQ ID NO: 214 - DNA, 321 bp, Artificial
  Synthetic
ggcatccagttgacccagtctccatccttcctgtctgcatctgtaggagacagagtcaccatcacttgccgggccagtcagggcatttacacttatttagcctggtatcagcaaaaaccagggaaagcccctaagctcctggtctatgttgcatccactttgcaaagtggggtcccatcaaggttcagcggcagtggatctgggacagaattcactctcacaatcagcagcctgcagcctgaagattttgcaacttattactgtcaacagcttaatagttaccctctcacttttggccaggggaccaagctggagatcaaa